European Patent Application EP 4 578 503 A2, published July 2, 2025. Title: NON-VIRAL IMMUNO-TARGETING. Applicant: University of Washington. Application EP. The sequence listing filed with the application follows.

SEQUENCE LISTING (95 sequences)

SEQ ID NO: 1 - protein, 36 aa, Homo sapiens
INAPQKVIEQSYNETWLGRQGPEGPSSIPPGTLTTL

SEQ ID NO: 2 - protein, 11 aa, Homo sapiens
GRQGPEGPSSI

SEQ ID NO: 3 - protein, 36 aa, Mus musculus
INAPQKVIEQSYNATWLGRQGPGGPDSIPQGTLTTL

SEQ ID NO: 4 - protein, 11 aa, Mus musculus
GRQGPGGPDSI

SEQ ID NO: 5 - protein, 3685 aa, Homo sapiens
MLWWEEVEDCYEREDVQKKTFTKWVNAQFSKFGKQHIENLFSDLQDGRRLLDLLEGLTGQKLPKEKGSTRVHALNNVNKALRVLQNNNVDLVNIGSTDIVDGNHKLTLGLIWNIILHWQVKNVMKNIMAGLQQTNSEKILLSWVRQSTRNYPQVNVINFTTSWSDGLALNALIHSHRPDLFDWNSVVCQQSATQRLEHAFNIARYQLGIEKLLDPEDVDTTYPDKKSILMYITSLFQVLPQQVSIEAIQEVEMLPRPPKVTKEEHFQLHHQMHYSQQITVSLAQGYERTSSPKPRFKSYAYTQAAYVTTSDPTRSPFPSQHLEAPEDKSFGSSLMESEVNLDRYQTALEEVLSWLLSAEDTLQAQGEISNDVEVVKDQFHTHEGYMMDLTAHQGRVGNILQLGSKLIGTGKLSEDEETEVQEQMNLLNSRWECLRVASMEKQSNLHRVLMDLQNQKLKELNDWLTKTEERTRKMEEEPLGPDLEDLKRQVQQHKVLQEDLEQEQVRVNSLTHMVVVVDESSGDHATAALEEQLKVLGDRWANICRWTEDRWVLLQDILLKWQRLTEEQCLFSAWLSEKEDAVNKIHTTGFKDQNEMLSSLQKLAVLKADLEKKKQSMGKLYSLKQDLLSTLKNKSVTQKTEAWLDNFARCWDNLVQKLEKSTAQISQAVTTTQPSLTQTTVMETVTTVTTREQILVKHAQEELPPPPPQKKRQITVDSEIRKRLDVDITELHSWITRSEAVLQSPEFAIFRKEGNFSDLKEKVNAIEREKAEKFRKLQDASRSAQALVEQMVNEGVNADSIKQASEQLNSRWIEFCQLLSERLNWLEYQNNIIAFYNQLQQLEQMTTTAENWLKIQPTTPSEPTAIKSQLKICKDEVNRLSGLQPQIERLKIQSIALKEKGQGPMFLDADFVAFTNHFKQVFSDVQAREKELQTIFDTLPPMRYQETMSAIRTWVQQSETKLSIPQLSVTDYEIMEQRLGELQALQSSLQEQQSGLYYLSTTVKEMSKKAPSEISRKYQSEFEEIEGRWKKLSSQLVEHCQKLEEQMNKLRKIQNHIQTLKKWMAEVDVFLKEEWPALGDSEILKKQLKQCRLLVSDIQTIQPSLNSVNEGGQKIKNEAEPEFASRLETELKELNTQWDHMCQQVYARKEALKGGLEKTVSLQKDLSEMHEWMTQAEEEYLERDFEYKTPDELQKAVEEMKRAKEEAQQKEAKVKLLTESVNSVIAQAPPVAQEALKKELETLTTNYQWLCTRLNGKCKTLEEVWACWHELLSYLEKANKWLNEVEFKLKTTENIPGGAEEISEVLDSLENLMRHSEDNPNQIRILAQTLTDGGVMDELINEELETFNSRWRELHEEAVRRQKLLEQSIQSAQETEKSLHLIQESLTFIDKQLAAYIADKVDAAQMPQEAQKIQSDLTSHEISLEEMKKHNQGKEAAQRVLSQIDVAQKKLQDVSMKFRLFQKPANFELRLQESKMILDEVKMHLPALETKSVEQEVVQSQLNHCVNLYKSLSEVKSEVEMVIKTGRQIVQKKQTENPKELDERVTALKLHYNELGAKVTERKQQLEKCLKLSRKMRKEMNVLTEWLAATDMELTKRSAVEGMPSNLDSEVAWGKATQKEIEKQKVHLKSITEVGEALKTVLGKKETLVEDKLSLLNSNWIAVTSRAEEWLNLLLEYQKHMETFDQNVDHITKWIIQADTLLDESEKKKPQQKEDVLKRLKAELNDIRPKVDSTRDQAANLMANRGDHCRKLVEPQISELNHRFAAISHRIKTGKASIPLKELEQFNSDIQKLLEPLEAEIQQGVNLKEEDFNKDMNEDNEGTVKELLQRGDNLQQRITDERKREEIKIKQQLLQTKHNALKDLRSQRRKKALEISHQWYQYKRQADDLLKCLDDIEKKLASLPEPRDERKIKEIDRELQKKKEELNAVRRQAEGLSEDGAAMAVEPTQIQLSKRWREIESKFAQFRRLNFAQIHTVREETMMVMTEDMPLEISYVPSTYLTEITHVSQALLEVEQLLNAPDLCAKDFEDLFKQEESLKNIKDSLQQSSGRIDIIHSKKTAALQSATPVERVKLQEALSQLDFQWEKVNKMYKDRQGRFDRSVEKWRRFHYDIKIFNQWLTEAEQFLRKTQIPENWEHAKYKWYLKELQDGIGQRQTVVRTLNATGEEIIQQSSKTDASILQEKLGSLNLRWQEVCKQLSDRKKRLEEQKNILSEFQRDLNEFVLWLEEADNIASIPLEPGKEQQLKEKLEQVKLLVEELPLRQGILKQLNETGGPVLVSAPISPEEQDKLENKLKQTNLQWIKVSRALPEKQGEIEAQIKDLGQLEKKLEDLEEQLNHLLLWLSPIRNQLEIYNQPNQEGPFDVQETEIAVQAKQPDVEEILSKGQHLYKEKPATQPVKRKLEDLSSEWKAVNRLLQELRAKQPDLAPGLTTIGASPTQTVTLVTQPVVTKETAISKLEMPSSLMLEVPALADFNRAWTELTDWLSLLDQVIKSQRVMVGDLEDINEMIIKQKATMQDLEQRRPQLEELITAAQNLKNKTSNQEARTIITDRIERIQNQWDEVQEHLQNRRQQLNEMLKDSTQWLEAKEEAEQVLGQARAKLESWKEGPYTVDAIQKKITETKQLAKDLRQWQTNVDVANDLALKLLRDYSADDTRKVHMITENINASWRSIHKRVSEREAALEETHRLLQQFPLDLEKFLAWLTEAETTANVLQDATRKERLLEDSKGVKELMKQWQDLQGEIEAHTDVYHNLDENSQKILRSLEGSDDAVLLQRRLDNMNFKWSELRKKSLNIRSHLEASSDQWKRLHLSLQELLVWLQLKDDELSRQAPIGGDFPAVQKQNDVHRAFKRELKTKEPVIMSTLETVRIFLTEQPLEGLEKLYQEPRELPPEERAQNVTRLLRKQAEEVNTEWEKLNLHSADWQRKIDETLERLQELQEATDELDLKLRQAEVIKGSWQPVGDLLIDSLQDHLEKVKALRGEIAPLKENVSHVNDLARQLTTLGIQLSPYNLSTLEDLNTRWKLLQVAVEDRVRQLHEAHRDFGPASQHFLSTSVQGPWERAISPNKVPYYINHETQTTCWDHPKMTELYQSLADLNNVRFSAYRTAMKLRRLQKALCLDLLSLSAACDALDQHNLKQNDQPMDILQIINCLTTIYDRLEQEHNNLVNVPLCVDMCLNWLLNVYDTGRTGRIRVLSFKTGIISLCKAHLEDKYRYLFKQVASSTGFCDQRRLGLLLHDSIQIPRQLGEVASFGGSNIEPSVRSCFQFANNKPEIEAALFLDWMRLEPQSMVWLPVLHRVAAAETAKHQAKCNICKECPIIGFRYRSLKHFNYDICQSCFFSGRVAKGHKMHYPMVEYCTPTTSGEDVRDFAKVLKNKFRTKRYFAKHPRMGYLPVQTVLEGDNMETPVTLINFWPVDSAPASSPQLSHDDTHSRIEHYASRLAEMENSNGSYLNDSISPNESIDDEHLLIQHYCQSLNQDSPLSQPRSPAQILISLESEERGELERILADLEEENRNLQAEYDRLKQQHEHKGLSPLPSPPEMMPTSPQSPRDAELIAEAKLLRQHKGRLEARMQILEDHNKQLESQLHRLRQLLEQPQAEAKVNGTTVSSPSTSLQRSDSSQPMLLRVVGSQTSDSMGEEDLLSPPQDTSTGLEEVMEQLNNSFPSSRGRNTPGKPMREDTM

SEQ ID NO: 6 - protein, 3678 aa, Mus musculus
MLWWEEVEDCYEREDVQKKTFTKWINAQFSKFGKQHIDNLFSDLQDGKRLLDLLEGLTGQKLPKEKGSTRVHALNNVNKALRVLQKNNVDLVNIGSTDIVDGNHKLTLGLIWNIILHWQVKNVMKTIMAGLQQTNSEKILLSWVRQSTRNYPQVNVINFTSSWSDGLALNALIHSHRPDLFDWNSVVSQHSATQRLEHAFNIAKCQLGIEKLLDPEDVATTYPDKKSILMYITSLFQVLPQQVSIEAIQEVEMLPRTSSKVTREEHFQLHHQMHYSQQITVSLAQGYEQTSSSPKPRFKSYAFTQAAYVATSDSTQSPYPSQHLEAPRDKSLDSSLMETEVNLDSYQTALEEVLSWLLSAEDTLRAQGEISNDVEEVKEQFHAHEGFMMDLTSHQGLVGNVLQLGSQLVGKGKLSEDEEAEVQEQMNLLNSRWECLRVASMEKQSKLHKVLMDLQNQKLKELDDWLTKTEERTKKMEEEPFGPDLEDLKCQVQQHKVLQEDLEQEQVRVNSLTHMVVVVDESSGDHATAALEEQLKVLGDRWANICRWTEDRWIVLQDILLKWQHFTEEQCLFSTWLSEKEDAMKNIQTSGFKDQNEMMSSLHKISTLKIDLEKKKPTMEKLSSLNQDLLSALKNKSVTQKMEIWMENFAQRWDNLTQKLEKSSAQISQAVTTTQPSLTQTTVMETVTMVTTREQIMVKHAQEELPPPPPQKKRQITVDSELRKRLDVDITELHSWITRSEAVLQSSEFAVYRKEGNISDLQEKVNAIAREKAEKFRKLQDASRSAQALVEQMANEGVNAESIRQASEQLNSRWTEFCQLLSERVNWLEYQTNIITFYNQLQQLEQMTTTAENLLKTQSTTLSEPTAIKSQLKICKDEVNRLSALQPQIEQLKIQSLQLKEKGQGPMFLDADFVAFTNHFNHIFDGVRAKEKELQTIFDTLPPMRYQETMSSIRTWIQQSESKLSVPYLSVTEYEIMEERLGKLQALQSSLKEQQNGFNYLSDTVKEMAKKAPSEICQKYLSEFEEIEGHWKKLSSQLVESCQKLEEHMNKLRKFQNHIKTLQKWMAEVDVFLKEEWPALGDAEILKKQLKQCRLLVGDIQTIQPSLNSVNEGGQKIKSEAELEFASRLETELRELNTQWDHICRQVYTRKEALKAGLDKTVSLQKDLSEMHEWMTQAEEEYLERDFEYKTPDELQTAVEEMKRAKEEALQKETKVKLLTETVNSVIAHAPPSAQEALKKELETLTTNYQWLCTRLNGKCKTLEEVWACWHELLSYLEKANKWLNEVELKLKTMENVPAGPEEITEVLESLENLMHHSEENPNQIRLLAQTLTDGGVMDELINEELETFNSRWRELHEEAVRKQKLLEQSIQSAQEIEKSLHLIQESLEFIDKQLAAYITDKVDAAQMPQEAQKIQSDLTSHEISLEEMKKHNQGKDANQRVLSQIDVAQKKLQDVSMKFRLFQKPANFEQRLEESKMILDEVKMHLPALETKSVEQEVIQSQLSHCVNLYKSLSEVKSEVEMVIKTGRQIVQKKQTENPKELDERVTALKLHYNELGAKVTERKQQLEKCLKLSRKMRKEMNVLTEWLAATDTELTKRSAVEGMPSNLDSEVAWGKATQKEIEKQKAHLKSVTELGESLKMVLGKKETLVEDKLSLLNSNWIAVTSRVEEWLNLLLEYQKHMETFDQNIEQITKWIIHADELLDESEKKKPQQKEDILKRLKAEMNDMRPKVDSTRDQAAKLMANRGDHCRKVVEPQISELNRRFAAISHRIKTGKASIPLKELEQFNSDIQKLLEPLEAEIQQGVNLKEEDFNKDMSEDNEGTVNELLQRGDNLQQRITDERKREEIKIKQQLLQTKHNALKDLRSQRRKKALEISHQWYQYKRQADDLLKCLDEIEKKLASLPEPRDERKLKEIDRELQKKKEELNAVRRQAEGLSENGAAMAVEPTQIQLSKRWRQIESNFAQFRRLNFAQIHTLHEETMVVTTEDMPLDVSYVPSTYLTEISHILQALSEVDHLLNTPELCAKDFEDLFKQEESLKNIKDNLQQISGRIDIIHKKKTAALQSATSMEKVKVQEAVAQMDFQGEKLHRMYKERQGRFDRSVEKWRHFHYDMKVFNQWLNEVEQFFKKTQNPENWEHAKYKWYLKELQDGIGQRQAVVRTLNATGEEIIQQSSKTDVNILQEKLGSLSLRWHDICKELAERRKRIEEQKNVLSEFQRDLNEFVLWLEEADNIAITPLGDEQQLKEQLEQVKLLAEELPLRQGILKQLNETGGAVLVSAPIRPEEQDKLEKKLKQTNLQWIKVSRALPEKQGELEVHLKDFRQLEEQLDHLLLWLSPIRNQLEIYNQPSQAGPFDIKEIEVTVHGKQADVERLLSKGQHLYKEKPSTQPVKRKLEDLRSEWEAVNHLLRELRTKQPDRAPGLSTTGASASQTVTLVTQSVVTKETVISKLEMPSSLLLEVPALADFNRAWTELTDWLSLLDRVIKSQRVMVGDLEDINEMIIKQKATLQDLEQRRPQLEELITAAQNLKNKTSNQEARTIITDRIERIQIQWDEVQEQLQNRRQQLNEMLKDSTQWLEAKEEAEQVIGQVRGKLDSWKEGPHTVDAIQKKITETKQLAKDLRQRQISVDVANDLALKLLRDYSADDTRKVHMITENINTSWGNIHKRVSEQEAALEETHRLLQQFPLDLEKFLSWITEAETTANVLQDASRKEKLLEDSRGVRELMKPWQDLQGEIETHTDIYHNLDENGQKILRSLEGSDEAPLLQRRLDNMNFKWSELQKKSLNIRSHLEASSDQWKRLHLSLQELLVWLQLKDDELSRQAPIGGDFPAVQKQNDIHRAFKRELKTKEPVIMSTLETVRIFLTEQPLEGLEKLYQEPRELPPEERAQNVTRLLRKQAEEVNAEWDKLNLRSADWQRKIDEALERLQELQEAADELDLKLRQAEVIKGSWQPVGDLLIDSLQDHLEKVKALRGEIAPLKENVNRVNDLAHQLTTLGIQLSPYNLSTLEDLNTRWRLLQVAVEDRVRQLHEAHRDFGPASQHFLSTSVQGPWERAISPNKVPYYINHETQTTCWDHPKMTELYQSLADLNNVRFSAYRTAMKLRRLQKALCLDLLSLSAACDALDQHNLKQNDQPMDILQIINCLTTIYDRLEQEHNNLVNVPLCVDMCLNWLLNVYDTGRTGRIRVLSFKTGIISLCKAHLEDKYRYLFKQVASSTGFCDQRRLGLLLHDSIQIPRQLGEVASFGGSNIEPSVRSCFQFANNKPEIEAALFLDWMRLEPQSMVWLPVLHRVAAAETAKHQAKCNICKECPIIGFRYRSLKHFNYDICQSCFFSGRVAKGHKMHYPMVEYCTPTTSGEDVRDFAKVLKNKFRTKRYFAKHPRMGYLPVQTVLEGDNMETPVTLINFWPVDSAPASSPQLSHDDTHSRIEHYASRLAEMENSNGSYLNDSISPNESIDDEHLLIQHYCQSLNQDSPLSQPRSPAQILISLESEERGELERILADLEEENRNLQAEYDRLKQQHEHKGLSPLPSPPEMMPTSPQSPRDAELIAEAKLLRQHKGRLEARMQILEDHNKQLESQLHRLRQLLEQPQAEAKVNGTTVSSPSTSLQRSDSSQPMLLRVVGSQTSESMGEEDLLSPPQDTSTGLEEVMEQLNNSFPSSRGRNAPGKPMREDTM

SEQ ID NO: 7 - protein, 3699 aa, Rattus norvegicus
MEDEREDVQKKTFTKWINAQFSKFGKQHIDNLFSDLQDGKRLLDLLEGLTGQKLPKEKGSTRVHALNNVNKALQVLQKNNVDLVNIGSTDIVDGNHKLTLGLIWNIILHWQVKNVMKTIMAGLQQTNSEKILLSWVRESTRNYPQVNVLNFTSSWSDGLALNALIHSHRPDLFDWNSVVSQQSATQRLEHAFNIAKCQLGIEKLLDPEDVATTYPDKKSILMYITSLFQVLPQQVSIEAIREVEMLPRPSKVTREEHFQLHHQMHYSQQITVSLAQGYEQTSSSPKPRFKSYAFTQAAYVATSDSSQSPYPSQHLEAPGSKSFGSSLIETEVNLDSYQTALEEVLSWLLSAEDTLRAQGEISKDVEEVKEQFHAHEGFMMDLTSHQGLVGNVLQLGSRLVGKGKLTEDEETEVQEQMNLLNSRWECLRVASMEKQSNLHKVLMDLQNQKLKELDDWLTKTEERTKKMEEEPLGPDLEDLKCQVQQHKVLQEDLEQEQVRVNSLTHMVVVVDESSGDHATAALEEQLKVLGDRWANICKWTEDRWILLQDILLKWQRFTEEQCLFSKWLSEKEDAMKNIQTSGFEDQNEMVSSLQNISALKIDLEKKKQSMEKLSSLNQDLLSALKNKSVTQKMEMWMENFAQRWDNLTQKLEKSSAQISQAVTTTQPSLTQTTVMETVTMVTTREQIMVKHAQEELPPPPPQKKRQITVDSEIRKRLDVDITELHSWITRSEAVLQSSEFAVYRKEGNISDLKEKVNAIAREKAEKFRKLQDASRSAQALVEQMVNEGVNAESIRQASEQLNSRWTEFCQLLSERVNWLEYQNNIITFYNQLQQLEQMTTTAENLLKTQPTTLSEPTAIKSQLKICKDEVNRLSALQPQIERLKIQSLTLKEKGQGPMFLDADFVAFTNHFNYVFDGVRAREKELQTIFDTLPPMRYQETMSSIRTWIQQSENKLSIPHLSVTEYEIMEERLGKLQALQSSLKEQQNGFNYLNATVKEIAKKAPSEISQKYQSEFEEVEGRWKKLSTQLVEHCQKLEEHMNKLRKFQNHKKTLQKWMAEVDVFLKEEWPALGDAEILKKQLKQCRLLVGDIQTIQPSLNSVNEGGQKIKSEAEFEFASRLEKELKELNTQWDHICRQVYTRKEALKAGLDKTVSLQKDLSEMHEWMTQAEEEYLERDFEYKTPDELQTAVEEMKRAKEEALQKEAKVKLLTETVNSVISQAPPAAQEALKKELETLTTNYQWLCTRLNGKCKTLEEVWACWHELLSYLEKANKWLNEVELKLKATENVPAGAEEITEVLESLENLMHHSEENPNQIRLLAQTLTDGGVMDELINEELETFNSRWRELHEEAVRKQKLLEQSIQSAQEIEKSLHLIQESLEFIDKQLAAYIADKVDAAQMPQEAQKIQSDLTSHEISLEEMKKHNQGKDANQRVLSQIDVAQKKLQDVSIKFRLFQKPANFEQRLEESKMILDEVKMHLPALETKSVEQEVVQSQLSHCVNLYKSLSEVKSEVEMVIKTGRQIVQKKQTENPKELDERVTALKLHYNELGAKVTERKQQLEKCLKLSRKMRKEMNVLTEWLAATDTELTKRSAVEGMPSNLDSEVAWGKATQKEIEKQKAHLKSVTELGDSLKTVLGKKETLVEDKLTLLNSNWIAVTSRVEEWLNLLLEYQKHMESFDQNVEHITKWIIHTDELLDESEKRKPQQKEDILKRLKAEMNDIRPKVDATRDQAAKLMANRGDYCRKIVEPQISELNRRFAAISHRIKTGKASIPLKELEQFNSDIQKLLEPLEAEIQQGVNLKEEDFNKDMSEDNEGTVNELLQRGDNLQQRITDERKREEIKLKQQLLQTKHNALKDLRSQRRKKALEISHQWYQYKSQADDLLKCLDEIEKKLASLPEPRDERKIKEIDRELQKKKEELNAVRRQAESLSENGAAMAVEPTQIQLSKRWREIESNFAQFRRLNFAQIHTLHEETMVVTTEDMPLDVSYVPSTYLTEISHILQALSEVEQLLNAPELNAKDFEDLFKQEESLKNIKENLQQISGRIDVIHKKKTAALQSATPMERVKLQEAVSQMDFHWEKLNRMYKERQGRFDRSVEKWRHFHYDMKVFNQWLNDVEQFFKKTQNPENWEHAKYKWYLKELQDGIGQRQAVVRTLNATGEEIIQQSSKTDANILQEKLGSLSLRWHEVCKELAERRKRVEEQKNVFSEFQRDLNEFVSWLEEADNIATTPPGDEEQLKEKLEQVKLLTEELPLRQGILKQLNETGGAVLVSAPIRPEEQDKLEKKLKQTNLQWIKVSRALPEKQGELEVHIKDFRQFEEQLDHLLLWLSPIRNQLEIYNQPSQPGPFDLKETEVTVQAKQPDVERLLSKGQHLYKEKPSTQPVKRKLEDLRSEWEAVNHLLWELRTKQPDRAPGLSTTGASASQTVTVVTQPVDTKETVISKLEMPSSLLLEVPALADFNRAWTELTDWLSLLDRVIKSQRVMVGDLEDINEMIIKQKLVESMMNSHLQGATLQDLEQRRPQLEELITAAQNLKNKTSNQEARTIITDRIERIQIQWDEVQEQLQNRRQQLNEMLKDSTQWLEAKEEAEQVIGQARGKLDSWKEGPHTMDAIQKKITETKQLAKDLRQRQINVDVANDLALKLLRDYSADDTRKVHMITENINTSWGNILKRVSEREAALEETQRLLQQFPLDLEKFLAWITEAETTANVLQDASRKEKLLEDSRGVRELMKPWQDLQGEIEAHTDIYHNLDENGQKILRSLEGSDEAPLLQRRLDNMNFKWSELRKKSLNIRSHLEVSSDQWKRLHLSLQELLVWLQLKDDELSRQAPIGGDFPAVQKQNDVHRAFKRELKTKEPVIMSTLETVRIFLTEQPLEGLEKLYQEPRELPPEERAQNVTRLLRKQAEEVNTEWDKLNLHSADWQRKIDEALERLQELQEAADELDLKLRQAEVIKGSWQPVGDLLIDSLQDHLEKVKALRGEIAPLKENVNHVNDLAHHLTTLGIQLSPYNLSILEDLNTRWRLLQVAVEDRVRQLHEAHRDFGPASQHFLSTSVQGPWERAISPNKVPYYINHETQTTCWDHPKMTELYQSLADLNNVRFSAYRTAMKLRRLQKALCLDLLSLSAACDALDQHNLKQNDQPMDILQIINCLTTIYDRLEQEHNNLVNVPLCVDMCLNWLLNVYDTGRTGRIRVLSFKTGIISLCKAHLEDKYRYLFKQVASSTGFCDQRRLGLLLHDSIQIPRQLGEVASFGGSNIEPSVRSCFQFANNKPEIEAALFLDWMRLEPQSMVWLPVLHRVAAAETAKHQAKCNICKECPIIGFRYRSLKHFNYDICQSCFFSGRVAKGHKMHYPMVEYCTPTTSGEDVRDFAKVLKNKFRTKRYFAKHPRMGYLPVQTVLEGDNMETPVTLINFWPVDSAPASSPQLSHDDTHSRIEHYASRLAEMENSNGSYLNDSISPNESIDDEHLLIQHYCQSLNQDSPLSQPRSPAQILISLESEERGELERILADLEEENRNLQAEYDRLKQQHEHKGLSPLPSPPEMMPTSPQSPRDAELIAEAKLLRQHKGRLEARMQILEDHNKQLESQLHRLRQLLEQPQAEAKVNGTTVSSPSTSLQRSDSSQPMLLRVVGSQTSESMGEEDLLSPPQDTSTGLEEVMEQLNNSFPSSRGHNVGSLFHMADDLGRAMESLVSVMIDEEGAE

SEQ ID NO: 8 - protein, 3677 aa, Oryctolagus cuniculus
  SITE 2570: note = misc_feature - Xaa can be any naturally occurring amino acid
  SITE 2597: note = misc_feature - Xaa can be any naturally occurring amino acid
MLWWEEVEDCYEREDVQKKTFTKWINAQFSKFGKQHIENLFSDLQDGRRLLDLLEGLTGQQLPKEKGSTRVHALNNVNKALRVLQKNNVDLVNIGSTDIVDGNHKLTLGLIWNIILHWQVKNVMKNIMAGLQQTNSEKILLSWVRQSTRNYSQVNVINFTTSWSDGLALNALIHSHRPDLFDWNSVVCQQSATQRLEHAFNIAKCQLGIEKLLDPEDVATTYPDKKSILMYITSLFQVLPQQVSIEAIQEVELLPRPSKVTREEHFQLHHQMHYSQQITVSLAQGYERTSSPKPRFKSYAYTQAAYVSTSDPTRSPFPSQHLEAPGDKSFGSSLMETEVSLDSYQTALEEVLSWLLSAEDTLQAQKEISSDVEEVKEQFHTHEGYMMDLTSHQGRVGNVLQLGSQLIRTGKLSEEEETEVQEQMNLLNSRWECLRVASMEKQSNLHKVLMDLQNQKLKELNDWLTKTEERTRKMEEEPLGPDLEDLKRQVQQHKVLQEDLEQEQVRVNSLTHMVVVVDESSGEHATAALEEQLKVLGDRWANICRWTEDRWVLLQDILLKWQRFTEEQCLFSTWLSEKEDAVNKIHTTGFKDQNEMLSSLHKLTVLKTDLEKKKQSMDKLSSLNQALLSTLKNKSVTQKMEAWLENFALRWDNLVQKLEKSSAQISQAVTTTQPSLTQTTVMETVTMVTTREQILVKHAQEELPPPPPQKKRQIIVDSEIRKRLDVDITELHSWITRSEAVLQSPEFAIYRKEGNFSDLKEKVNAIEREKAEKFRKLQDASRSAQALVEQMVNEGVNADSIKQALEQLNSRWIEFCQLLSERLHWLEYQNSIITFYNQLQQLEQMITTAENWLKTQPTTASEPTAIKSQLKMCKDEVNRLSALQPQIERLKIQSTALKEKGQGPMFLDADFVAFTNHFNQVFADAQAREKELQTIFDTLPPTRYQETISTIRTWIQQSEPKLSIPQLSVTEYEIMEQRLGELQALQSSLQEQQSGLTYLSTTVKEMAKKAPSEISRKYQSEFEEIEGHWKKLSYQLVDHCQKLEEQMNKLRKIQNHIKTLKKWMAEVDVFLKEEWPALGDSEILKKQLKQCRLLVNDIQTIQPSLNSVNESGQKIKNEAEPEFASRLETELRELNSQWDHMCRQVYTRKDALKAGLDKTLSLQKDLSEMHEWMTQAEEEYLERDFEYKTPDELQTAVEEMKRAKEEAQQKESKVKLLTESVNSVIAQAPPAAQEALKKELDTLTTNYQWLCTRLNGKCKTLEEVWACWHELLSYLEKANKWLNEVEVKLKTTETLPGGAEEISEVLDSLENLMQHSEDNPNQIRILAQTLTDGGVMDELINEELETFNSRWRELHEEAVRRQKLLEQSIQSAQEIEKSLHLIQESLAFIDKQLAAYIADKVDAAQMPQEAQKIQSDLTSHEISLEEMKKHNQGKEAAQRVLSQIDVAQKKLQDVSMKFRLFQKPANFEQRLEESKMILDEVKMHLPALETKSVEQEVVQSQLNHCVNLYKSLSEVKSEVEMVIKTGRQIVQKKQTENPKELDERVTALKLHYNELGAKVTERKQQLEKCLKLSRKMRKEMNALTEWLAATDMELTKRSAVEGMPSNLDAEIAWGKATQKEVEKQKAHLKSVIELGEALKTVLGKKETLVEDKLSLLNSNWVAVTSRAEEWLNLLLEYQKHMETFDQNVDHITKWIIQADTLLDESEKKKPQQKEDVLKRLKAEMNDIRPKVDSIRDQAANLMANRGDHCRKVVEPKISELNHRFAAISHRIKTGKASIPLKELEQFNSDIQKLLEPLEAEIQQGVNLKEEDFNKDMSEDNEGTVKELLQRGDNLHERITDERKREEIKIKQQLLQTKHNALKDLRSQRRKKALEISHQWYQYKRQADDLLKCLDDIEKKLASLPDPKDERKIKEIDRELQKKKEELNAVHRQAEGLSEDGAAMAVEPIQIQLSKRWREIESKFAQFRRLNFAQIHTVREETMVVMTEDMPLEISYVPSTYLTEITHVSQALSEVDQLLNAPDLSAKDFEDLFKQEESLKNIKECMQQISGRIDVIHNKKAAALQSATAAERVKLQEALAQLDSQWEKVNKMYKDRQGRFDRSVEKWRRFHYDMKIFNQWLTEAEQFLKKTQIPENWEHAKYKWYLKELQDGIGQRQTVVRTLNTTGEEIIQQSSKTDANILQEKLGNLNLRWQEVCKQLAERRKRLEEQKNILSEFQRDLNEFVLWLEEADNITSIPLEPGNEQQLKEKLEQVKLLAEELPLRQGILKQLNEAGGTALVSAPISPEEQDKLENKLKQTNLQWIKVSKALPEKQEEIVAHVKELGQLEEQLNHLLLWLTPIRNQLEIYNQPNQTGPFDIKETEVAVQAKQPDVERILSKGQHLYKEKPATQPVKRKLEDLSSEWKVVNYLLQELRAKRPDLPPGPATIGASPSQTVTLVTQTVVTKEISLSELEMPSSLLLEVPALADFNRAWTELTDWLSLLDRVLKSQQVIVGDLEDINEMIIKQKATLQELEQRRPQLEELITAAQNLKNKTSNQEARTIITDRIERIQNQWDEVQEHLQNRSSSLNXMLKDSTQWLEAKEELSSLGQARAKLSXMEEGPYPMNALQKKIEETKQLAKDLRQWQINVDVANDLALKLLRDYSADDTRKVHMITENINASWGSIHKRVNEREATLEEAYRLLQQFPLDLEKFLAWLTEAETTANVLQDATHKERLPEDSKGVRELMKQWQDLQGEIEAHTDIYHNLDENGQKILRSLEGSDEAVLLQRRLDNMNFKWSELRKKSLNIRSHLEASSDQWKRLHLSLQELLVWLQLKDDELNRQAPVGGDFPAVQKQNDVHRAFKRELKTKEPVIMSTLETVRIFLTEQPLGGLEKLYQEPRELPPDERAQNVTRLLRKQAEEVNAEWEKLNLHSTDWQRKLDEALERLQELQEATDELDLKLRQAEVIKGSWQPVGDLLIDSLQDHLEKVKALRGEIAPLKENVSHVNDLGRQLTTLGIQLSPYNLSTLEDLNTRWKLLQVAVEDRIRQLHEAHRDFGPASQHFLSTSVQGPWERAISPNKVPYYINHETQTTCWDHPKMTELYQSLADLNNVRFSAYRTAMKLRRLQKALCLDLLTLSAACDALDQHNLKQNDQPMDILQIINCLTTVYDRLEQEHNNLVNVPLCVDMCLNWLLNVYDTGRTGRIRVLSFKTGIISLCKAHLEDKYRYLFKQVASSTGFCDQRRLGLLLHDSIQIPRQLGEVASFGGSNIEPSVRSCFQFANNKPEIEAALFLDWMRLEPQSMVWLPVLHRVAAAETAKHQAKCNICKECPIIGFRYRSLKHFNYDICQSCFFSGRVAKGHKMHYPMVEYCTPTTSGEDVRDFAKVLKNKFRTKRYFAKHPRMGYLPVQTVLEGDNMETPVTLINFWPVDSAPASSPQLSHDDTHSRIEHYASRLAEMENSNGSYLNDSISPNESIDDEHLLIQHYCQSLNQDSPLSQPRSPAQILISLESEERGELERILADLEEENRNLQAEYDRLKQQHEHKGLSPLPSPPEMMPTSPQSPRDAELIAEAKLLRQHKGRLEARMQILEDHNKQLESQLHRLRQLLEQPQAEAKVNGTTVSSPSTSLQRSDSSQPMLLRVVGSQTSESMGEEDLPSPPQDTSTGLEEVMEQLNNSFPSSRGRNTPGKPMREDTM

SEQ ID NO: 9 - protein, 14 aa, synthetic construct
  REGION 1..14: note = Synthetic
AEEQKLISEEDLLK

SEQ ID NO: 10 - protein, 5 aa, synthetic construct
  REGION 1..5: note = Synthetic
DDAMH

SEQ ID NO: 11 - protein, 5 aa, synthetic construct
  REGION 1..5: note = Synthetic
DYSMH

SEQ ID NO: 12 - protein, 5 aa, synthetic construct
  REGION 1..5: note = Synthetic
EYTIH

SEQ ID NO: 13 - protein, 5 aa, synthetic construct
  REGION 1..5: note = Synthetic
DYSMH

SEQ ID NO: 14 - protein, 5 aa, synthetic construct
  REGION 1..5: note = Synthetic
DFSMH

SEQ ID NO: 15 - protein, 5 aa, synthetic construct
  REGION 1..5: note = Synthetic
AYSMH

SEQ ID NO: 16 - protein, 5 aa, synthetic construct
  REGION 1..5: note = Synthetic
DYSMH

SEQ ID NO: 17 - protein, 5 aa, synthetic construct
  REGION 1..5: note = Synthetic
DYSMH

SEQ ID NO: 18 - protein, 17 aa, synthetic construct
  REGION 1..17: note = Synthetic
WINTETGEPTYADDFKG

SEQ ID NO: 19 - protein, 17 aa, synthetic construct
  REGION 1..17: note = Synthetic
WINTETGEPTYADDFKG

SEQ ID NO: 20 - protein, 17 aa, synthetic construct
  REGION 1..17: note = Synthetic
GINCNSGGTSYTQKFKD

SEQ ID NO: 21 - protein, 17 aa, synthetic construct
  REGION 1..17: note = Synthetic
WINTETGEPTYADDFKG

SEQ ID NO: 22 - protein, 17 aa, synthetic construct
  REGION 1..17: note = Synthetic
WINTETGDPTYADDFKG

SEQ ID NO: 23 - protein, 17 aa, synthetic construct
  REGION 1..17: note = Synthetic
WINTETGEATYADDFKG

SEQ ID NO: 24 - protein, 17 aa, synthetic construct
  REGION 1..17: note = Synthetic
WINTETGEPTYADDFKG

SEQ ID NO: 25 - protein, 17 aa, synthetic construct
  REGION 1..17: note = Synthetic
WINTETGEPTYADDFKG

SEQ ID NO: 26 - skipped

SEQ ID NO: 27 - protein, 5 aa, synthetic construct
  REGION 1..5: note = Synthetic
GASGY

SEQ ID NO: 28 - protein, 11 aa, synthetic construct
  REGION 1..11: note = Synthetic
RFFYGSSQFAY

SEQ ID NO: 29 - protein, 4 aa, synthetic construct
  REGION 1..4: note = Synthetic
RGEF

SEQ ID NO: 30 - protein, 4 aa, synthetic construct
  REGION 1..4: note = Synthetic
RGDY

SEQ ID NO: 31 - protein, 4 aa, synthetic construct
  REGION 1..4: note = Synthetic
RGDY

SEQ ID NO: 32 - protein, 4 aa, synthetic construct
  REGION 1..4: note = Synthetic
RGDY

SEQ ID NO: 33 - protein, 5 aa, synthetic construct
  REGION 1..5: note = Synthetic
GRSAY

SEQ ID NO: 34 - protein, 16 aa, synthetic construct
  REGION 1..16: note = Synthetic
RSSQSLVHSNGKTYLH

SEQ ID NO: 35 - protein, 11 aa, synthetic construct
  REGION 1..11: note = Synthetic
KASQSVSKNVA

SEQ ID NO: 36 - protein, 15 aa, synthetic construct
  REGION 1..15: note = Synthetic
RASKSVTTSGYSYMH

SEQ ID NO: 37 - protein, 11 aa, synthetic construct
  REGION 1..11: note = Synthetic
KASQSVNKNVA

SEQ ID NO: 38 - protein, 16 aa, synthetic construct
  REGION 1..16: note = Synthetic
RSSQSLVHSNRNIYLH

SEQ ID NO: 39 - protein, 16 aa, synthetic construct
  REGION 1..16: note = Synthetic
RSSQSLVRSNRNIYLH

SEQ ID NO: 40 - protein, 16 aa, synthetic construct
  REGION 1..16: note = Synthetic
RSSQSLVHNNRNIYLH

SEQ ID NO: 41 - protein, 11 aa, synthetic construct
  REGION 1..11: note = Synthetic
KASQTVSNNVA

SEQ ID NO: 42 - protein, 7 aa, synthetic construct
  REGION 1..7: note = Synthetic
KVSNRFS

SEQ ID NO: 43 - protein, 7 aa, synthetic construct
  REGION 1..7: note = Synthetic
SSSKRYS

SEQ ID NO: 44 - protein, 7 aa, synthetic construct
  REGION 1..7: note = Synthetic
LASNLES

SEQ ID NO: 45 - protein, 7 aa, synthetic construct
  REGION 1..7: note = Synthetic
SASKRYT

SEQ ID NO: 46 - protein, 7 aa, synthetic construct
  REGION 1..7: note = Synthetic
KVSNRFS

SEQ ID NO: 47 - protein, 7 aa, synthetic construct
  REGION 1..7: note = Synthetic
KVSNRFS

SEQ ID NO: 48 - protein, 7 aa, synthetic construct
  REGION 1..7: note = Synthetic
KVSNRFS

SEQ ID NO: 49 - protein, 7 aa, synthetic construct
  REGION 1..7: note = Synthetic
SASNRYT

SEQ ID NO: 50 - protein, 9 aa, synthetic construct
  REGION 1..9: note = Synthetic
SQSTHVPWT

SEQ ID NO: 51 - protein, 9 aa, synthetic construct
  REGION 1..9: note = Synthetic
HQDYNSPWT

SEQ ID NO: 52 - protein, 9 aa, synthetic construct
  REGION 1..9: note = Synthetic
QHSRELPLT

SEQ ID NO: 53 - protein, 9 aa, synthetic construct
  REGION 1..9: note = Synthetic
LQDYTSPWT

SEQ ID NO: 54 - protein, 9 aa, synthetic construct
  REGION 1..9: note = Synthetic
SQDKYIPWT

SEQ ID NO: 55 - protein, 9 aa, synthetic construct
  REGION 1..9: note = Synthetic
SQDSHIPWT

SEQ ID NO: 56 - protein, 9 aa, synthetic construct
  REGION 1..9: note = Synthetic
SQDRYIPWT

SEQ ID NO: 57 - protein, 9 aa, synthetic construct
  REGION 1..9: note = Synthetic
QQDYSSPWT

SEQ ID NO: 58 - protein, 5 aa, synthetic construct
  REGION 1..5: note = Synthetic
TYGMS

SEQ ID NO: 59 - protein, 5 aa, synthetic construct
  REGION 1..5: note = Synthetic
TYGMT

SEQ ID NO: 60 - protein, 17 aa, synthetic construct
  REGION 1..17: note = Synthetic
WINTSSGVPTYADDFKG

SEQ ID NO: 61 - protein, 17 aa, synthetic construct
  REGION 1..17: note = Synthetic
WINTYSGVPTYANDFKG

SEQ ID NO: 62 - protein, 17 aa, synthetic construct
  REGION 1..17: note = Synthetic
WINTYSGLPTYTNDFKG

SEQ ID NO: 63 - protein, 17 aa, synthetic construct
  REGION 1..17: note = Synthetic
WINTYSGLPTYADDFKG

SEQ ID NO: 64 - protein, 17 aa, synthetic construct
  REGION 1..17: note = Synthetic
WINTYSGVPTYADDFKG

SEQ ID NO: 65 - protein, 17 aa, synthetic construct
  REGION 1..17: note = Synthetic
WINTFSGVPTYTDDFKG

SEQ ID NO: 66 - protein, 10 aa, synthetic construct
  REGION 1..10: note = Synthetic
PIHMVVAEDY

SEQ ID NO: 67 - protein, 10 aa, synthetic construct
  REGION 1..10: note = Synthetic
PIHKVVAEDY

SEQ ID NO: 68 - protein, 10 aa, synthetic construct
  REGION 1..10: note = Synthetic
PITTVVPFDY

SEQ ID NO: 69 - protein, 10 aa, synthetic construct
  REGION 1..10: note = Synthetic
PITTVVPFDY

SEQ ID NO: 70 - protein, 10 aa, synthetic construct
  REGION 1..10: note = Synthetic
PITKVVAGDF

SEQ ID NO: 71 - protein, 10 aa, synthetic construct
  REGION 1..10: note = Synthetic
PITTVVPFDY

SEQ ID NO: 72 - protein, 17 aa, synthetic construct
  REGION 1..17: note = Synthetic
KSSQILLYGRNQKNYLA

SEQ ID NO: 73 - protein, 17 aa, synthetic construct
  REGION 1..17: note = Synthetic
RSSQSLLYSGNQKNYLA

SEQ ID NO: 74 - protein, 16 aa, synthetic construct
  REGION 1..16: note = Synthetic
RSSQSLVYTYGNTYLH

SEQ ID NO: 75 - protein, 16 aa, synthetic construct
  REGION 1..16: note = Synthetic
RSSQSLVYNYGNTYLH

SEQ ID NO: 76 - protein, 17 aa, synthetic construct
  REGION 1..17: note = Synthetic
KSSQSLLYRSNQKNYLA

SEQ ID NO: 77 - protein, 16 aa, synthetic construct
  REGION 1..16: note = Synthetic
RSSQSLVYSTGNTYLH

SEQ ID NO: 78 - protein, 7 aa, synthetic construct
  REGION 1..7: note = Synthetic
WASTRES

SEQ ID NO: 79 - protein, 7 aa, synthetic construct
  REGION 1..7: note = Synthetic
WASTWES

SEQ ID NO: 80 - protein, 7 aa, synthetic construct
  REGION 1..7: note = Synthetic
KVSNRFS

SEQ ID NO: 81 - protein, 7 aa, synthetic construct
  REGION 1..7: note = Synthetic
KVSNRFS

SEQ ID NO: 82 - protein, 7 aa, synthetic construct
  REGION 1..7: note = Synthetic
WASTRES

SEQ ID NO: 83 - protein, 7 aa, synthetic construct
  REGION 1..7: note = Synthetic
KVSNRFS

SEQ ID NO: 84 - protein, 9 aa, synthetic construct
  REGION 1..9: note = Synthetic
QQYYSKPYT

SEQ ID NO: 85 - protein, 9 aa, synthetic construct
  REGION 1..9: note = Synthetic
QQYYTFPYT

SEQ ID NO: 86 - protein, 9 aa, synthetic construct
  REGION 1..9: note = Synthetic
SQSRHSPWT

SEQ ID NO: 87 - protein, 9 aa, synthetic construct
  REGION 1..9: note = Synthetic
SQSRHSPWT

SEQ ID NO: 88 - protein, 9 aa, synthetic construct
  REGION 1..9: note = Synthetic
QQYFSSPYT

SEQ ID NO: 89 - protein, 9 aa, synthetic construct
  REGION 1..9: note = Synthetic
SQSRHGPWT

SEQ ID NO: 90 - skipped

SEQ ID NO: 91 - protein, 17 aa, synthetic construct
  REGION 1..17: note = Synthetic
  SITE 6: note = MISC_FEATURE - Xaa at position 6 is Ser or Thr
  SITE 8: note = MISC_FEATURE - Xaa at position 8 is Asp or Glu
  SITE 9: note = MISC_FEATURE - Xaa at position 9 is any amino acid
  SITE 10: note = MISC_FEATURE - Xaa at position 10 is Thr or Ser
WINTEXGXXXYADDFKG

SEQ ID NO: 92-94 - skipped (3 entries)

SEQ ID NO: 95 - protein, 7 aa, synthetic construct
  REGION 1..7: note = Synthetic
  SITE 3: note = MISC_FEATURE - Xaa at position 3 is any amino acid
  SITE 4: note = MISC_FEATURE - Xaa at position 4 is any amino acid
  SITE 5: note = MISC_FEATURE - Xaa at position 5 is any amino acid
QDXXXPT